European Patent Specification EP 3 976 054 B1, published January 7, 2026. Title: TIMED ADMINISTRATION OF DECITABINE AND 5-AZACYTIDINE FOR CANCER TREATMENT. Applicant: THE CLEVELAND CLINIC FOUNDATION. The sequence listing filed with the application follows.

SEQUENCE LISTING (10 sequences)

SEQ ID NO: 1 - DNA, 22 bp, Artificial sequence
  DNA Primer
ctgacttctacactgagcatgg

SEQ ID NO: 2 - DNA, 22 bp, Artificial sequence
  DNA Primer
cacgcattgacaggttaatcac

SEQ ID NO: 3 - DNA, 21 bp, Artificial sequence
  DNA Primer
aagggtacaaggatttcaggg

SEQ ID NO: 4 - DNA, 21 bp, Artificial sequence
  DNA Primer
acaatatacgtaccatccggc

SEQ ID NO: 5 - DNA, 18 bp, Artificial sequence
  DNA Primer
aagctgcccgtctttctc

SEQ ID NO: 6 - DNA, 21 bp, Artificial sequence
  DNA Primer
accacttcccaatcttcacac

SEQ ID NO: 7 - DNA, 21 bp, Artificial sequence
  DNA Primer
atccccgtgtatgactttgtc

SEQ ID NO: 8 - DNA, 21 bp, Artificial sequence
  DNA Primer
cttcatctggaacaggtctcg

SEQ ID NO: 9 - DNA, 19 bp, Artificial sequence
  DNA Primer
acatcgctcagacaccatg

SEQ ID NO: 10 - DNA, 22 bp, Artificial sequence
  DNA Primer
tgtagttgaggtcaatgaaggg